European Patent Application EP 4 800 015 A1, published September 2, 2026. Title: AZABICYCLIO DERIVATIVE AND PREPARATION METHOD THEREFOR, AND USE. Applicant: ZHEJIANG HISUN PHARMACEUTICAL CO., LTD. Application CN. The sequence listing filed with the application follows.

SEQUENCE LISTING (1 sequence)

SEQ ID NO: 1 - DNA, 45 bp, synthetic construct
  source 1..45: mol_type = other DNA
ttttttttttttttttttttttccaagtaaaacgacggccagtgc